European Patent Application EP 4 674 841 A2, published January 7, 2026. Title: PHARMACEUTICAL COMPOUND. Applicant: DUKE STREET BIO LIMITED. Application EP, filed February 14, 2023. The sequence listing filed with the application follows.

SEQUENCE LISTING (3 sequences)

SEQ ID NO: 1 - DNA, 30 bp, synthetic construct
  source 1..30: mol_type = other DNA
  modified_base 15: mod_base = OTHER; note = deoxyuridine
accctgctgtgggcnggagaacaaggtgat

SEQ ID NO: 2 - DNA, 31 bp, synthetic construct
  source 1..31: mol_type = other DNA
atcaccttgttctccahgcccacagcagggt

SEQ ID NO: 3 - DNA, 29 bp, synthetic construct
  source 1..29: mol_type = other DNA
accctgctgtgggcggagaacaaggtgat